European Patent Application EP 4 803 104 A1, published September 9, 2026. Title: 금속 나노 입자-핵산 결합체를 기반으로 하는 운반체를 포함하는 대사성 질환 치료제. Applicant: NES BIOTECHNOLOGY. The sequence listing filed with the application follows.

SEQUENCE LISTING (15 sequences)

SEQ ID NO: 1 - DNA, 75 bp, synthetic construct
  source 1..75: mol_type = other DNA
aactagagaacccactgcttactggcgccgccaccatggccctgtggatgcgcctcctgcccctgctggcgctgc

SEQ ID NO: 2 - DNA, 51 bp, synthetic construct
  source 1..51: mol_type = other DNA
cagatggctggcaactagaaggcacagtcgctagttgcagtagttctccag

SEQ ID NO: 3 - DNA, 56 bp, synthetic construct
  source 1..56: mol_type = other DNA
aactagagaacccactgcttactggcgccgccaccatggccctgtggatgcgcctc

SEQ ID NO: 4 - DNA, 81 bp, synthetic construct
  source 1..81: mol_type = other DNA
agggcccccgcccagctccacctgccccacctgcaggtcctctgcctcccgcttggtcctgggtgtgtagaagaagcctcg

SEQ ID NO: 5 - DNA, 84 bp, synthetic construct
  source 1..84: mol_type = other DNA
gtggagctgggcgggggccctggtgcaggcagcctgcagcccttggccctggaggggtcccggcagaagcgtggcattgtggaa

SEQ ID NO: 6 - DNA, 35 bp, synthetic construct
  source 1..35: mol_type = other DNA
cagatatacgcgttgacattgattattgactagtt

SEQ ID NO: 7 - DNA, 35 bp, synthetic construct
  source 1..35: mol_type = other DNA
tttccgcctcagaagaaaatacagcatagcaaaac

SEQ ID NO: 8 - DNA, 36 bp, synthetic construct
  source 1..36: mol_type = other DNA
gatccaccggtcgccaccatggccctgtggatgcgc

SEQ ID NO: 9 - DNA, 52 bp, synthetic construct
  source 1..52: mol_type = other DNA
taagcttggatcctctagagcggccgctctagttgcagtagttctccagctg

SEQ ID NO: 10 - DNA, 20 bp, synthetic construct
  source 1..20: mol_type = other DNA
  misc_feature 1..5: note = Thiolated base
cttagggttaggcgttttgc

SEQ ID NO: 11 - DNA, 21 bp, synthetic construct
  source 1..21: mol_type = other DNA
  misc_feature 1..5: note = Thiolated base
ctacagggcgcgtggggatac

SEQ ID NO: 12 - DNA, 5770 bp, synthetic construct
  source 1..5770: mol_type = other DNA
gacggatcgggagatctcccgatcccctatggtgcactctcagtacaatctgctctgatgccgcatagttaagccagtatctgctccctgcttgtgtgttggaggtcgctgagtagtgcgcgagcaaaatttaagctacaacaaggcaaggcttgaccgacaattgcatgaagaatctgcttagggttaggcgttttgcgctgcttcgcgatgtacgggccagatatacgcgttgacattgattattgactagttattaatagtaatcaattacggggtcattagttcatagcccatatatggagttccgcgttacataacttacggtaaatggcccgcctggctgaccgcccaacgacccccgcccattgacgtcaataatgacgtatgttcccatagtaacgccaatagggactttccattgacgtcaatgggtggagtatttacggtaaactgcccacttggcagtacatcaagtgtatcatatgccaagtacgccccctattgacgtcaatgacggtaaatggcccgcctggcattatgcccagtacatgaccttatgggactttcctacttggcagtacatctacgtattagtcatcgctattaccatggtgatgcggttttggcagtacatcaatgggcgtggatagcggtttgactcacggggatttccaagtctccaccccattgacgtcaatgggagtttgttttggcaccaaaatcaacgggactttccaaaatgtcgtaacaactccgccccattgacgcaaatgggcggtaggcgtgtacggtgggaggtctatataagcagagctctctggctaactagagaacccactgcttactggcgccgccaccatggccctgtggatgcgcctcctgcccctgctggcgctgctggccctctggggacctgacccagccgcagcctttgtgaaccaacacctgtgcggctcacacctggtggaagctctctacctagtgtgcggggaacgaggcttcttctacacacccaagacccgccgggaggcagaggacctgcaggtggggcaggtggagctgggcgggggccctggtgcaggcagcctgcagcccttggccctggaggggtccctgcagaagcgtggcattgtggaacaatgctgtaccagcatctgctccctctaccagctggagaactactgcaactagcgactgtgccttctagttgccagccatctgttgtttgcccctcccccgtgccttccttgaccctggaaggtgccactcccactgtcctttcctaataaaatgaggaaattgcatcgcattgtctgagtaggtgtcattctattctggggggtggggtggggcaggacagcaagggggaggattgggaagacaatagcaggcatgctggggatgcggtgggctctatggcttctgaggcggaaagaaccagctggggctctagggggtatccccacgcgccctgtagcggcgcattaagcgcggcgggtgtggtggttacgcgcagcgtgaccgctacacttgccagcgccctagcgcccgctcctttcgctttcttcccttcctttctcgccacgttcgccggctttccccgtcaagctctaaatcgggggctccctttagggttccgatttagtgctttacggcacctcgaccccaaaaaacttgattagggtgatggttcacgtagtgggccatcgccctgatagacggtttttcgccctttgacgttggagtccacgttctttaatagtggactcttgttccaaactggaacaacactcaaccctatctcggtctattcttttgatttataagggattttgccgatttcggcctattggttaaaaaatgagctgatttaacaaaaatttaacgcgaattaattctgtggaatgtgtgtcagttagggtgtggaaagtccccaggctccccagcaggcagaagtatgcaaagcatgcatctcaattagtcagcaaccaggtgtggaaagtccccaggctccccagcaggcagaagtatgcaaagcatgcatctcaattagtcagcaaccatagtcccgcccctaactccgcccatcccgcccctaactccgcccagttccgcccattctccgccccatggctgactaattttttttatttatgcagaggccgaggccgcctctgcctctgagctattccagaagtagtgaggaggcttttttggaggcctaggcttttgcaaaaagctcccgggagcttgtatatccattttcggatctgatcagcacgtgatgaaaaagcctgaactcaccgcgacgtctgtcgagaagtttctgatcgaaaagttcgacagcgtctccgacctgatgcagctctcggagggcgaagaatctcgtgctttcagcttcgatgtaggagggcgtggatatgtcctgcgggtaaatagctgcgccgatggtttctacaaagatcgttatgtttatcggcactttgcatcggccgcgctcccgattccggaagtgcttgacattggggaattcagcgagagcctgacctattgcatctcccgccgtgcacagggtgtcacgttgcaagacctgcctgaaaccgaactgcccgctgttctgcagccggtcgcggaggccatggatgcgatcgctgcggccgatcttagccagacgagcgggttcggcccattcggaccgcaaggaatcggtcaatacactacatggcgtgatttcatatgcgcgattgctgatccccatgtgtatcactggcaaactgtgatggacgacaccgtcagtgcgtccgtcgcgcaggctctcgatgagctgatgctttgggccgaggactgccccgaagtccggcacctcgtgcacgcggatttcggctccaacaatgtcctgacggacaatggccgcataacagcggtcattgactggagcgaggcgatgttcggggattcccaatacgaggtcgccaacatcttcttctggaggccgtggttggcttgtatggagcagcagacgcgctacttcgagcggaggcatccggagcttgcaggatcgccgcggctccgggcgtatatgctccgcattggtcttgaccaactctatcagagcttggttgacggcaatttcgatgatgcagcttgggcgcagggtcgatgcgacgcaatcgtccgatccggagccgggactgtcgggcgtacacaaatcgcccgcagaagcgcggccgtctggaccgatggctgtgtagaagtactcgccgatagtggaaaccgacgccccagcactcgtccgagggcaaaggaatagcacgtgctacgagatttcgattccaccgccgccttctatgaaaggttgggcttcggaatcgttttccgggacgccggctggatgatcctccagcgcggggatctcatgctggagttcttcgcccaccccaacttgtttattgcagcttataatggttacaaataaagcaatagcatcacaaatttcacaaataaagcatttttttcactgcattctagttgtggtttgtccaaactcatcaatgtatcttatcatgtctgtataccgtcgacctctagctagagcttggcgtaatcatggtcatagctgtttcctgtgtgaaattgttatccgctcacaattccacacaacatacgagccggaagcataaagtgtaaagcctggggtgcctaatgagtgagctaactcacattaattgcgttgcgctcactgcccgctttccagtcgggaaacctgtcgtgccagctgcattaatgaatcggccaacgcgcggggagaggcggtttgcgtattgggcgctcttccgcttcctcgctcactgactcgctgcgctcggtcgttcggctgcggcgagcggtatcagctcactcaaaggcggtaatacggttatccacagaatcaggggataacgcaggaaagaacatgtgagcaaaaggccagcaaaaggccaggaaccgtaaaaaggccgcgttgctggcgtttttccataggctccgcccccctgacgagcatcacaaaaatcgacgctcaagtcagaggtggcgaaacccgacaggactataaagataccaggcgtttccccctggaagctccctcgtgcgctctcctgttccgaccctgccgcttaccggatacctgtccgcctttctcccttcgggaagcgtggcgctttctcatagctcacgctgtaggtatctcagttcggtgtaggtcgttcgctccaagctgggctgtgtgcacgaaccccccgttcagcccgaccgctgcgccttatccggtaactatcgtcttgagtccaacccggtaagacacgacttatcgccactggcagcagccactggtaacaggattagcagagcgaggtatgtaggcggtgctacagagttcttgaagtggtggcctaactacggctacactagaagaacagtatttggtatctgcgctctgctgaagccagttaccttcggaaaaagagttggtagctcttgatccggcaaacaaaccaccgctggtagcggtggtttttttgtttgcaagcagcagattacgcgcagaaaaaaaggatctcaagaagatcctttgatcttttctacggggtctgacgctcagtggaacgaaaactcacgttaagggattttggtcatgagattatcaaaaaggatcttcacctagatccttttaaattaaaaatgaagttttaaatcaatctaaagtatatatgagtaaacttggtctgacagttaccaatgcttaatcagtgaggcacctatctcagcgatctgtctatttcgttcatccatagttgcctgactccccgtcgtgtagataactacgatacgggagggcttaccatctggccccagtgctgcaatgataccgcgagacccacgctcaccggctccagatttatcagcaataaaccagccagccggaagggccgagcgcagaagtggtcctgcaactttatccgcctccatccagtctattaattgttgccgggaagctagagtaagtagttcgccagttaatagtttgcgcaacgttgttgccattgctacaggcatcgtggtgtcacgctcgtcgtttggtatggcttcattcagctccggttcccaacgatcaaggcgagttacatgatcccccatgttgtgcaaaaaagcggttagctccttcggtcctccgatcgttgtcagaagtaagttggccgcagtgttatcactcatggttatggcagcactgcataattctcttactgtcatgccatccgtaagatgcttttctgtgactggtgagtactcaaccaagtcattctgagaatagtgtatgcggcgaccgagttgctcttgcccggcgtcaatacgggataataccgcgccacatagcagaactttaaaagtgctcatcattggaaaacgttcttcggggcgaaaactctcaaggatcttaccgctgttgagatccagttcgatgtaacccactcgtgcacccaactgatcttcagcatcttttactttcaccagcgtttctgggtgagcaaaaacaggaaggcaaaatgccgcaaaaaagggaataagggcgacacggaaatgttgaatactcatactcttcctttttcaatattattgaagcatttatcagggttattgtctcatgagcggatacatatttgaatgtatttagaaaaataaacaaataggggttccgcgcacatttccccgaaaagtgccacctgacgtc

SEQ ID NO: 13 - DNA, 5770 bp, synthetic construct
  source 1..5770: mol_type = other DNA
gacggatcgggagatctcccgatcccctatggtgcactctcagtacaatctgctctgatgccgcatagttaagccagtatctgctccctgcttgtgtgttggaggtcgctgagtagtgcgcgagcaaaatttaagctacaacaaggcaaggcttgaccgacaattgcatgaagaatctgcttagggttaggcgttttgcgctgcttcgcgatgtacgggccagatatacgcgttgacattgattattgactagttattaatagtaatcaattacggggtcattagttcatagcccatatatggagttccgcgttacataacttacggtaaatggcccgcctggctgaccgcccaacgacccccgcccattgacgtcaataatgacgtatgttcccatagtaacgccaatagggactttccattgacgtcaatgggtggagtatttacggtaaactgcccacttggcagtacatcaagtgtatcatatgccaagtacgccccctattgacgtcaatgacggtaaatggcccgcctggcattatgcccagtacatgaccttatgggactttcctacttggcagtacatctacgtattagtcatcgctattaccatggtgatgcggttttggcagtacatcaatgggcgtggatagcggtttgactcacggggatttccaagtctccaccccattgacgtcaatgggagtttgttttggcaccaaaatcaacgggactttccaaaatgtcgtaacaactccgccccattgacgcaaatgggcggtaggcgtgtacggtgggaggtctatataagcagagctctctggctaactagagaacccactgcttactggcgccgccaccatggccctgtggatgcgcctcctgcccctgctggcgctgctggccctctggggacctgacccagccgcagcctttgtgaaccaacacctgtgcggctcacacctggtggaagctctctacctagtgtgcggggaacgaggcttcttctacacacccaggaccaagcgggaggcagaggacctgcaggtggggcaggtggagctgggcgggggccctggtgcaggcagcctgcagcccttggccctggaggggtcccggcagaagcgtggcattgtggaacaatgctgtaccagcatctgctccctctaccagctggagaactactgcaactagcgactgtgccttctagttgccagccatctgttgtttgcccctcccccgtgccttccttgaccctggaaggtgccactcccactgtcctttcctaataaaatgaggaaattgcatcgcattgtctgagtaggtgtcattctattctggggggtggggtggggcaggacagcaagggggaggattgggaagacaatagcaggcatgctggggatgcggtgggctctatggcttctgaggcggaaagaaccagctggggctctagggggtatccccacgcgccctgtagcggcgcattaagcgcggcgggtgtggtggttacgcgcagcgtgaccgctacacttgccagcgccctagcgcccgctcctttcgctttcttcccttcctttctcgccacgttcgccggctttccccgtcaagctctaaatcgggggctccctttagggttccgatttagtgctttacggcacctcgaccccaaaaaacttgattagggtgatggttcacgtagtgggccatcgccctgatagacggtttttcgccctttgacgttggagtccacgttctttaatagtggactcttgttccaaactggaacaacactcaaccctatctcggtctattcttttgatttataagggattttgccgatttcggcctattggttaaaaaatgagctgatttaacaaaaatttaacgcgaattaattctgtggaatgtgtgtcagttagggtgtggaaagtccccaggctccccagcaggcagaagtatgcaaagcatgcatctcaattagtcagcaaccaggtgtggaaagtccccaggctccccagcaggcagaagtatgcaaagcatgcatctcaattagtcagcaaccatagtcccgcccctaactccgcccatcccgcccctaactccgcccagttccgcccattctccgccccatggctgactaattttttttatttatgcagaggccgaggccgcctctgcctctgagctattccagaagtagtgaggaggcttttttggaggcctaggcttttgcaaaaagctcccgggagcttgtatatccattttcggatctgatcagcacgtgatgaaaaagcctgaactcaccgcgacgtctgtcgagaagtttctgatcgaaaagttcgacagcgtctccgacctgatgcagctctcggagggcgaagaatctcgtgctttcagcttcgatgtaggagggcgtggatatgtcctgcgggtaaatagctgcgccgatggtttctacaaagatcgttatgtttatcggcactttgcatcggccgcgctcccgattccggaagtgcttgacattggggaattcagcgagagcctgacctattgcatctcccgccgtgcacagggtgtcacgttgcaagacctgcctgaaaccgaactgcccgctgttctgcagccggtcgcggaggccatggatgcgatcgctgcggccgatcttagccagacgagcgggttcggcccattcggaccgcaaggaatcggtcaatacactacatggcgtgatttcatatgcgcgattgctgatccccatgtgtatcactggcaaactgtgatggacgacaccgtcagtgcgtccgtcgcgcaggctctcgatgagctgatgctttgggccgaggactgccccgaagtccggcacctcgtgcacgcggatttcggctccaacaatgtcctgacggacaatggccgcataacagcggtcattgactggagcgaggcgatgttcggggattcccaatacgaggtcgccaacatcttcttctggaggccgtggttggcttgtatggagcagcagacgcgctacttcgagcggaggcatccggagcttgcaggatcgccgcggctccgggcgtatatgctccgcattggtcttgaccaactctatcagagcttggttgacggcaatttcgatgatgcagcttgggcgcagggtcgatgcgacgcaatcgtccgatccggagccgggactgtcgggcgtacacaaatcgcccgcagaagcgcggccgtctggaccgatggctgtgtagaagtactcgccgatagtggaaaccgacgccccagcactcgtccgagggcaaaggaatagcacgtgctacgagatttcgattccaccgccgccttctatgaaaggttgggcttcggaatcgttttccgggacgccggctggatgatcctccagcgcggggatctcatgctggagttcttcgcccaccccaacttgtttattgcagcttataatggttacaaataaagcaatagcatcacaaatttcacaaataaagcatttttttcactgcattctagttgtggtttgtccaaactcatcaatgtatcttatcatgtctgtataccgtcgacctctagctagagcttggcgtaatcatggtcatagctgtttcctgtgtgaaattgttatccgctcacaattccacacaacatacgagccggaagcataaagtgtaaagcctggggtgcctaatgagtgagctaactcacattaattgcgttgcgctcactgcccgctttccagtcgggaaacctgtcgtgccagctgcattaatgaatcggccaacgcgcggggagaggcggtttgcgtattgggcgctcttccgcttcctcgctcactgactcgctgcgctcggtcgttcggctgcggcgagcggtatcagctcactcaaaggcggtaatacggttatccacagaatcaggggataacgcaggaaagaacatgtgagcaaaaggccagcaaaaggccaggaaccgtaaaaaggccgcgttgctggcgtttttccataggctccgcccccctgacgagcatcacaaaaatcgacgctcaagtcagaggtggcgaaacccgacaggactataaagataccaggcgtttccccctggaagctccctcgtgcgctctcctgttccgaccctgccgcttaccggatacctgtccgcctttctcccttcgggaagcgtggcgctttctcatagctcacgctgtaggtatctcagttcggtgtaggtcgttcgctccaagctgggctgtgtgcacgaaccccccgttcagcccgaccgctgcgccttatccggtaactatcgtcttgagtccaacccggtaagacacgacttatcgccactggcagcagccactggtaacaggattagcagagcgaggtatgtaggcggtgctacagagttcttgaagtggtggcctaactacggctacactagaagaacagtatttggtatctgcgctctgctgaagccagttaccttcggaaaaagagttggtagctcttgatccggcaaacaaaccaccgctggtagcggtggtttttttgtttgcaagcagcagattacgcgcagaaaaaaaggatctcaagaagatcctttgatcttttctacggggtctgacgctcagtggaacgaaaactcacgttaagggattttggtcatgagattatcaaaaaggatcttcacctagatccttttaaattaaaaatgaagttttaaatcaatctaaagtatatatgagtaaacttggtctgacagttaccaatgcttaatcagtgaggcacctatctcagcgatctgtctatttcgttcatccatagttgcctgactccccgtcgtgtagataactacgatacgggagggcttaccatctggccccagtgctgcaatgataccgcgagacccacgctcaccggctccagatttatcagcaataaaccagccagccggaagggccgagcgcagaagtggtcctgcaactttatccgcctccatccagtctattaattgttgccgggaagctagagtaagtagttcgccagttaatagtttgcgcaacgttgttgccattgctacaggcatcgtggtgtcacgctcgtcgtttggtatggcttcattcagctccggttcccaacgatcaaggcgagttacatgatcccccatgttgtgcaaaaaagcggttagctccttcggtcctccgatcgttgtcagaagtaagttggccgcagtgttatcactcatggttatggcagcactgcataattctcttactgtcatgccatccgtaagatgcttttctgtgactggtgagtactcaaccaagtcattctgagaatagtgtatgcggcgaccgagttgctcttgcccggcgtcaatacgggataataccgcgccacatagcagaactttaaaagtgctcatcattggaaaacgttcttcggggcgaaaactctcaaggatcttaccgctgttgagatccagttcgatgtaacccactcgtgcacccaactgatcttcagcatcttttactttcaccagcgtttctgggtgagcaaaaacaggaaggcaaaatgccgcaaaaaagggaataagggcgacacggaaatgttgaatactcatactcttcctttttcaatattattgaagcatttatcagggttattgtctcatgagcggatacatatttgaatgtatttagaaaaataaacaaataggggttccgcgcacatttccccgaaaagtgccacctgacgtc

SEQ ID NO: 14 - DNA, 6704 bp, synthetic construct
  source 1..6704: mol_type = other DNA
gacggatcgggagatctcccgatcccctatggtgcactctcagtacaatctgctctgatgccgcatagttaagccagtatctgctccctgcttgtgtgttggaggtcgctgagtagtgcgcgagcaaaatttaagctacaacaaggcaaggcttgaccgacaattgcatgaagaatctgcttagggttaggcgttttgcgctgcttcgcgatgtacgggccagatatacgcgttgacattgattattgactagttattaatagtaatcaattacggggtcattagttcatagcccatatatggagttccgcgttacataacttacggtaaatggcccgcctggctgaccgcccaacgacccccgcccattgacgtcaataatgacgtatgttcccatagtaacgccaatagggactttccattgacgtcaatgggtggagtatttacggtaaactgcccacttggcagtacatcaagtgtatcatatgccaagtacgccccctattgacgtcaatgacggtaaatggcccgcctggcattatgcccagtacatgaccttatgggactttcctacttggcagtacatctacgtattagtcatcgctattaccatggtgatgcggttttggcagtacatcaatgggcgtggatagcggtttgactcacggggatttccaagtctccaccccattgacgtcaatgggagtttgttttggcaccaaaatcaacgggactttccaaaatgtcgtaacaactccgccccattgacgcaaatgggcggtaggcgtgtacggtgggaggtctatataagcagagctcgtttagtgaaccgtcagatcgcctggagacgccatccacgctgttttgacctccatagaagacaccgggaccgatccagcctcccctcgaagctgatcctgagaacttcagggtgagtctatgggacccttgatgttttctttccccttcttttctatggttaagttcatgtcataggaaggggagaagtaacagggtacacatattgaccaaatcagggtaattttgcatttgtaattttaaaaaatgctttcttcttttaatatacttttttgtttatcttatttctaatactttccctaatctctttctttcagggcaataatgatacaatgtatcatgcctctttgcaccattctaaagaataacagtgataatttctgggttaaggcaatagcaatatttctgcatataaatatttctgcatataaattgtaactgatgtaagaggtttcatattgctaatagcagctacaatccagctaccattctgcttttattttatggttgggataaggctggattattctgagtccaagctaggcccttttgctaatcatgttcatacctcttatcttcctcccacagctcctgggcaacgtgctggtctgtgtgctggcccatcactttggcaaagaattccgcgggcccgggatccaccggtcgccaccatggccctgtggatgcgcctcctgcccctgctggcgctgctggccctctggggacctgacccagccgcagcctttgtgaaccaacacctgtgcggctcacacctggtggaagctctctacctagtgtgcggggaacgaggcttcttctacacacccaagacccgccgggaggcagaggacctgcaggtggggcaggtggagctgggcgggggccctggtgcaggcagcctgcagcccttggccctggaggggtccctgcagaagcgtggcattgtggaacaatgctgtaccagcatctgctccctctaccagctggagaactactgcaactagagcggccgctctagaggatccaagcttatcgataccgtcgacctcgagggcccagatctaattcaccccaccagtgcaggctgcctatcagaaagtggtggctggtgtggctaatgccctggcccacaagtatcactaagctcgctttcttgctgtccaatttctattaaaggttcctttgttccctaagtccaactactaaactgggggatattatgaagggccttgagcatctggattctgcctaataaaaaacatttattttcattgcaatgatgtatttaaattatttctgaatattttactaaaaagggaatgtgggaggtcagtgcatttaaaacataaagaaatgaagagctagttcaaaccttgggaaaatacactatatcttaaactccatgaaagaaggtgaggctgcaaacagctaatgcacattggcaacagcccctgatgcctatgccttattcatccctcagaaaaggattcaagtagaggcttgatttggaggttaaagttttgctatgctgtattttcttctgaggcggaaagaaccagctggggctctagggggtatccccacgcgccctgtagcggcgcattaagcgcggcgggtgtggtggttacgcgcagcgtgaccgctacacttgccagcgccctagcgcccgctcctttcgctttcttcccttcctttctcgccacgttcgccggctttccccgtcaagctctaaatcgggggctccctttagggttccgatttagtgctttacggcacctcgaccccaaaaaacttgattagggtgatggttcacgtagtgggccatcgccctgatagacggtttttcgccctttgacgttggagtccacgttctttaatagtggactcttgttccaaactggaacaacactcaaccctatctcggtctattcttttgatttataagggattttgccgatttcggcctattggttaaaaaatgagctgatttaacaaaaatttaacgcgaattaattctgtggaatgtgtgtcagttagggtgtggaaagtccccaggctccccagcaggcagaagtatgcaaagcatgcatctcaattagtcagcaaccaggtgtggaaagtccccaggctccccagcaggcagaagtatgcaaagcatgcatctcaattagtcagcaaccatagtcccgcccctaactccgcccatcccgcccctaactccgcccagttccgcccattctccgccccatggctgactaattttttttatttatgcagaggccgaggccgcctctgcctctgagctattccagaagtagtgaggaggcttttttggaggcctaggcttttgcaaaaagctcccgggagcttgtatatccattttcggatctgatcagcacgtgatgaaaaagcctgaactcaccgcgacgtctgtcgagaagtttctgatcgaaaagttcgacagcgtctccgacctgatgcagctctcggagggcgaagaatctcgtgctttcagcttcgatgtaggagggcgtggatatgtcctgcgggtaaatagctgcgccgatggtttctacaaagatcgttatgtttatcggcactttgcatcggccgcgctcccgattccggaagtgcttgacattggggaattcagcgagagcctgacctattgcatctcccgccgtgcacagggtgtcacgttgcaagacctgcctgaaaccgaactgcccgctgttctgcagccggtcgcggaggccatggatgcgatcgctgcggccgatcttagccagacgagcgggttcggcccattcggaccgcaaggaatcggtcaatacactacatggcgtgatttcatatgcgcgattgctgatccccatgtgtatcactggcaaactgtgatggacgacaccgtcagtgcgtccgtcgcgcaggctctcgatgagctgatgctttgggccgaggactgccccgaagtccggcacctcgtgcacgcggatttcggctccaacaatgtcctgacggacaatggccgcataacagcggtcattgactggagcgaggcgatgttcggggattcccaatacgaggtcgccaacatcttcttctggaggccgtggttggcttgtatggagcagcagacgcgctacttcgagcggaggcatccggagcttgcaggatcgccgcggctccgggcgtatatgctccgcattggtcttgaccaactctatcagagcttggttgacggcaatttcgatgatgcagcttgggcgcagggtcgatgcgacgcaatcgtccgatccggagccgggactgtcgggcgtacacaaatcgcccgcagaagcgcggccgtctggaccgatggctgtgtagaagtactcgccgatagtggaaaccgacgccccagcactcgtccgagggcaaaggaatagcacgtgctacgagatttcgattccaccgccgccttctatgaaaggttgggcttcggaatcgttttccgggacgccggctggatgatcctccagcgcggggatctcatgctggagttcttcgcccaccccaacttgtttattgcagcttataatggttacaaataaagcaatagcatcacaaatttcacaaataaagcatttttttcactgcattctagttgtggtttgtccaaactcatcaatgtatcttatcatgtctgtataccgtcgacctctagctagagcttggcgtaatcatggtcatagctgtttcctgtgtgaaattgttatccgctcacaattccacacaacatacgagccggaagcataaagtgtaaagcctggggtgcctaatgagtgagctaactcacattaattgcgttgcgctcactgcccgctttccagtcgggaaacctgtcgtgccagctgcattaatgaatcggccaacgcgcggggagaggcggtttgcgtattgggcgctcttccgcttcctcgctcactgactcgctgcgctcggtcgttcggctgcggcgagcggtatcagctcactcaaaggcggtaatacggttatccacagaatcaggggataacgcaggaaagaacatgtgagcaaaaggccagcaaaaggccaggaaccgtaaaaaggccgcgttgctggcgtttttccataggctccgcccccctgacgagcatcacaaaaatcgacgctcaagtcagaggtggcgaaacccgacaggactataaagataccaggcgtttccccctggaagctccctcgtgcgctctcctgttccgaccctgccgcttaccggatacctgtccgcctttctcccttcgggaagcgtggcgctttctcatagctcacgctgtaggtatctcagttcggtgtaggtcgttcgctccaagctgggctgtgtgcacgaaccccccgttcagcccgaccgctgcgccttatccggtaactatcgtcttgagtccaacccggtaagacacgacttatcgccactggcagcagccactggtaacaggattagcagagcgaggtatgtaggcggtgctacagagttcttgaagtggtggcctaactacggctacactagaagaacagtatttggtatctgcgctctgctgaagccagttaccttcggaaaaagagttggtagctcttgatccggcaaacaaaccaccgctggtagcggtggtttttttgtttgcaagcagcagattacgcgcagaaaaaaaggatctcaagaagatcctttgatcttttctacggggtctgacgctcagtggaacgaaaactcacgttaagggattttggtcatgagattatcaaaaaggatcttcacctagatccttttaaattaaaaatgaagttttaaatcaatctaaagtatatatgagtaaacttggtctgacagttaccaatgcttaatcagtgaggcacctatctcagcgatctgtctatttcgttcatccatagttgcctgactccccgtcgtgtagataactacgatacgggagggcttaccatctggccccagtgctgcaatgataccgcgagacccacgctcaccggctccagatttatcagcaataaaccagccagccggaagggccgagcgcagaagtggtcctgcaactttatccgcctccatccagtctattaattgttgccgggaagctagagtaagtagttcgccagttaatagtttgcgcaacgttgttgccattgctacaggcatcgtggtgtcacgctcgtcgtttggtatggcttcattcagctccggttcccaacgatcaaggcgagttacatgatcccccatgttgtgcaaaaaagcggttagctccttcggtcctccgatcgttgtcagaagtaagttggccgcagtgttatcactcatggttatggcagcactgcataattctcttactgtcatgccatccgtaagatgcttttctgtgactggtgagtactcaaccaagtcattctgagaatagtgtatgcggcgaccgagttgctcttgcccggcgtcaatacgggataataccgcgccacatagcagaactttaaaagtgctcatcattggaaaacgttcttcggggcgaaaactctcaaggatcttaccgctgttgagatccagttcgatgtaacccactcgtgcacccaactgatcttcagcatcttttactttcaccagcgtttctgggtgagcaaaaacaggaaggcaaaatgccgcaaaaaagggaataagggcgacacggaaatgttgaatactcatactcttcctttttcaatattattgaagcatttatcagggttattgtctcatgagcggatacatatttgaatgtatttagaaaaataaacaaataggggttccgcgcacatttccccgaaaagtgccacctgacgtc

SEQ ID NO: 15 - DNA, 6704 bp, synthetic construct
  source 1..6704: mol_type = other DNA
gacggatcgggagatctcccgatcccctatggtgcactctcagtacaatctgctctgatgccgcatagttaagccagtatctgctccctgcttgtgtgttggaggtcgctgagtagtgcgcgagcaaaatttaagctacaacaaggcaaggcttgaccgacaattgcatgaagaatctgcttagggttaggcgttttgcgctgcttcgcgatgtacgggccagatatacgcgttgacattgattattgactagttattaatagtaatcaattacggggtcattagttcatagcccatatatggagttccgcgttacataacttacggtaaatggcccgcctggctgaccgcccaacgacccccgcccattgacgtcaataatgacgtatgttcccatagtaacgccaatagggactttccattgacgtcaatgggtggagtatttacggtaaactgcccacttggcagtacatcaagtgtatcatatgccaagtacgccccctattgacgtcaatgacggtaaatggcccgcctggcattatgcccagtacatgaccttatgggactttcctacttggcagtacatctacgtattagtcatcgctattaccatggtgatgcggttttggcagtacatcaatgggcgtggatagcggtttgactcacggggatttccaagtctccaccccattgacgtcaatgggagtttgttttggcaccaaaatcaacgggactttccaaaatgtcgtaacaactccgccccattgacgcaaatgggcggtaggcgtgtacggtgggaggtctatataagcagagctcgtttagtgaaccgtcagatcgcctggagacgccatccacgctgttttgacctccatagaagacaccgggaccgatccagcctcccctcgaagctgatcctgagaacttcagggtgagtctatgggacccttgatgttttctttccccttcttttctatggttaagttcatgtcataggaaggggagaagtaacagggtacacatattgaccaaatcagggtaattttgcatttgtaattttaaaaaatgctttcttcttttaatatacttttttgtttatcttatttctaatactttccctaatctctttctttcagggcaataatgatacaatgtatcatgcctctttgcaccattctaaagaataacagtgataatttctgggttaaggcaatagcaatatttctgcatataaatatttctgcatataaattgtaactgatgtaagaggtttcatattgctaatagcagctacaatccagctaccattctgcttttattttatggttgggataaggctggattattctgagtccaagctaggcccttttgctaatcatgttcatacctcttatcttcctcccacagctcctgggcaacgtgctggtctgtgtgctggcccatcactttggcaaagaattccgcgggcccgggatccaccggtcgccaccatggccctgtggatgcgcctcctgcccctgctggcgctgctggccctctggggacctgacccagccgcagcctttgtgaaccaacacctgtgcggctcacacctggtggaagctctctacctagtgtgcggggaacgaggcttcttctacacacccaggaccaagcgggaggcagaggacctgcaggtggggcaggtggagctgggcgggggccctggtgcaggcagcctgcagcccttggccctggaggggtcccggcagaagcgtggcattgtggaacaatgctgtaccagcatctgctccctctaccagctggagaactactgcaactagagcggccgctctagaggatccaagcttatcgataccgtcgacctcgagggcccagatctaattcaccccaccagtgcaggctgcctatcagaaagtggtggctggtgtggctaatgccctggcccacaagtatcactaagctcgctttcttgctgtccaatttctattaaaggttcctttgttccctaagtccaactactaaactgggggatattatgaagggccttgagcatctggattctgcctaataaaaaacatttattttcattgcaatgatgtatttaaattatttctgaatattttactaaaaagggaatgtgggaggtcagtgcatttaaaacataaagaaatgaagagctagttcaaaccttgggaaaatacactatatcttaaactccatgaaagaaggtgaggctgcaaacagctaatgcacattggcaacagcccctgatgcctatgccttattcatccctcagaaaaggattcaagtagaggcttgatttggaggttaaagttttgctatgctgtattttcttctgaggcggaaagaaccagctggggctctagggggtatccccacgcgccctgtagcggcgcattaagcgcggcgggtgtggtggttacgcgcagcgtgaccgctacacttgccagcgccctagcgcccgctcctttcgctttcttcccttcctttctcgccacgttcgccggctttccccgtcaagctctaaatcgggggctccctttagggttccgatttagtgctttacggcacctcgaccccaaaaaacttgattagggtgatggttcacgtagtgggccatcgccctgatagacggtttttcgccctttgacgttggagtccacgttctttaatagtggactcttgttccaaactggaacaacactcaaccctatctcggtctattcttttgatttataagggattttgccgatttcggcctattggttaaaaaatgagctgatttaacaaaaatttaacgcgaattaattctgtggaatgtgtgtcagttagggtgtggaaagtccccaggctccccagcaggcagaagtatgcaaagcatgcatctcaattagtcagcaaccaggtgtggaaagtccccaggctccccagcaggcagaagtatgcaaagcatgcatctcaattagtcagcaaccatagtcccgcccctaactccgcccatcccgcccctaactccgcccagttccgcccattctccgccccatggctgactaattttttttatttatgcagaggccgaggccgcctctgcctctgagctattccagaagtagtgaggaggcttttttggaggcctaggcttttgcaaaaagctcccgggagcttgtatatccattttcggatctgatcagcacgtgatgaaaaagcctgaactcaccgcgacgtctgtcgagaagtttctgatcgaaaagttcgacagcgtctccgacctgatgcagctctcggagggcgaagaatctcgtgctttcagcttcgatgtaggagggcgtggatatgtcctgcgggtaaatagctgcgccgatggtttctacaaagatcgttatgtttatcggcactttgcatcggccgcgctcccgattccggaagtgcttgacattggggaattcagcgagagcctgacctattgcatctcccgccgtgcacagggtgtcacgttgcaagacctgcctgaaaccgaactgcccgctgttctgcagccggtcgcggaggccatggatgcgatcgctgcggccgatcttagccagacgagcgggttcggcccattcggaccgcaaggaatcggtcaatacactacatggcgtgatttcatatgcgcgattgctgatccccatgtgtatcactggcaaactgtgatggacgacaccgtcagtgcgtccgtcgcgcaggctctcgatgagctgatgctttgggccgaggactgccccgaagtccggcacctcgtgcacgcggatttcggctccaacaatgtcctgacggacaatggccgcataacagcggtcattgactggagcgaggcgatgttcggggattcccaatacgaggtcgccaacatcttcttctggaggccgtggttggcttgtatggagcagcagacgcgctacttcgagcggaggcatccggagcttgcaggatcgccgcggctccgggcgtatatgctccgcattggtcttgaccaactctatcagagcttggttgacggcaatttcgatgatgcagcttgggcgcagggtcgatgcgacgcaatcgtccgatccggagccgggactgtcgggcgtacacaaatcgcccgcagaagcgcggccgtctggaccgatggctgtgtagaagtactcgccgatagtggaaaccgacgccccagcactcgtccgagggcaaaggaatagcacgtgctacgagatttcgattccaccgccgccttctatgaaaggttgggcttcggaatcgttttccgggacgccggctggatgatcctccagcgcggggatctcatgctggagttcttcgcccaccccaacttgtttattgcagcttataatggttacaaataaagcaatagcatcacaaatttcacaaataaagcatttttttcactgcattctagttgtggtttgtccaaactcatcaatgtatcttatcatgtctgtataccgtcgacctctagctagagcttggcgtaatcatggtcatagctgtttcctgtgtgaaattgttatccgctcacaattccacacaacatacgagccggaagcataaagtgtaaagcctggggtgcctaatgagtgagctaactcacattaattgcgttgcgctcactgcccgctttccagtcgggaaacctgtcgtgccagctgcattaatgaatcggccaacgcgcggggagaggcggtttgcgtattgggcgctcttccgcttcctcgctcactgactcgctgcgctcggtcgttcggctgcggcgagcggtatcagctcactcaaaggcggtaatacggttatccacagaatcaggggataacgcaggaaagaacatgtgagcaaaaggccagcaaaaggccaggaaccgtaaaaaggccgcgttgctggcgtttttccataggctccgcccccctgacgagcatcacaaaaatcgacgctcaagtcagaggtggcgaaacccgacaggactataaagataccaggcgtttccccctggaagctccctcgtgcgctctcctgttccgaccctgccgcttaccggatacctgtccgcctttctcccttcgggaagcgtggcgctttctcatagctcacgctgtaggtatctcagttcggtgtaggtcgttcgctccaagctgggctgtgtgcacgaaccccccgttcagcccgaccgctgcgccttatccggtaactatcgtcttgagtccaacccggtaagacacgacttatcgccactggcagcagccactggtaacaggattagcagagcgaggtatgtaggcggtgctacagagttcttgaagtggtggcctaactacggctacactagaagaacagtatttggtatctgcgctctgctgaagccagttaccttcggaaaaagagttggtagctcttgatccggcaaacaaaccaccgctggtagcggtggtttttttgtttgcaagcagcagattacgcgcagaaaaaaaggatctcaagaagatcctttgatcttttctacggggtctgacgctcagtggaacgaaaactcacgttaagggattttggtcatgagattatcaaaaaggatcttcacctagatccttttaaattaaaaatgaagttttaaatcaatctaaagtatatatgagtaaacttggtctgacagttaccaatgcttaatcagtgaggcacctatctcagcgatctgtctatttcgttcatccatagttgcctgactccccgtcgtgtagataactacgatacgggagggcttaccatctggccccagtgctgcaatgataccgcgagacccacgctcaccggctccagatttatcagcaataaaccagccagccggaagggccgagcgcagaagtggtcctgcaactttatccgcctccatccagtctattaattgttgccgggaagctagagtaagtagttcgccagttaatagtttgcgcaacgttgttgccattgctacaggcatcgtggtgtcacgctcgtcgtttggtatggcttcattcagctccggttcccaacgatcaaggcgagttacatgatcccccatgttgtgcaaaaaagcggttagctccttcggtcctccgatcgttgtcagaagtaagttggccgcagtgttatcactcatggttatggcagcactgcataattctcttactgtcatgccatccgtaagatgcttttctgtgactggtgagtactcaaccaagtcattctgagaatagtgtatgcggcgaccgagttgctcttgcccggcgtcaatacgggataataccgcgccacatagcagaactttaaaagtgctcatcattggaaaacgttcttcggggcgaaaactctcaaggatcttaccgctgttgagatccagttcgatgtaacccactcgtgcacccaactgatcttcagcatcttttactttcaccagcgtttctgggtgagcaaaaacaggaaggcaaaatgccgcaaaaaagggaataagggcgacacggaaatgttgaatactcatactcttcctttttcaatattattgaagcatttatcagggttattgtctcatgagcggatacatatttgaatgtatttagaaaaataaacaaataggggttccgcgcacatttccccgaaaagtgccacctgacgtc